European Patent Application EP 4 180 455 A1, published May 17, 2023. Title: Method for selectively manufacturing antibody-drug conjugate. Applicant: Daiichi Sankyo Company, Limited. Application EP. The sequence listing filed with the application follows.

SEQUENCE LISTING (34 sequences)

SEQ ID NO: 1 - DNA, 1410 bp, synthetic construct
  misc_feature 1..1410: note = hTINA1-H1
  source 1..1410: mol_type = other DNA
  CDS 1..1410: protein_id = 2; translation = MKHLWFFLLLVAAPRWVLSQVQLVQSGAEVKKPGASVKVSCKASGYTFTTAGMQWVRQAPGQGLEWMGWINTHSGVPKYAEDFKGRVTISADTSTSTAYLQLSSLKSEDTAVYYCARSGFGSSYWYFDVWGQGTLVTVSSASTKGPSVFPLAPSSKSTSGGTAALGCLVKDYFPEPVTVSWNSGALTSGVHTFPAVLQSSGLYSLSSVVTVPSSSLGTQTYICNVNHKPSNTKVDKRVEPKSCDKTHTCPPCPAPELLGGPSVFLFPPKPKDTLMISRTPEVTCVVVDVSHEDPEVKFNWYVDGVEVHNAKTKPREEQYNSTYRVVSVLTVLHQDWLNGKEYKCKVSNKALPAPIEKTISKAKGQPREPQVYTLPPSREEMTKNQVSLTCLVKGFYPSDIAVEWESNGQPENNYKTTPPVLDSDGSFFLYSKLTVDKSRWQQGNVFSCSVMHEALHNHYTQKSLSLSPGK
atgaaacacctgtggttcttcctcctgctggtggcagctcccagatgggtgctgagccaggtgcagctggtgcagtctggcgccgaagtgaagaaaccaggcgccagcgtgaaggtgtcctgcaaggccagcggctacacctttaccaccgccggcatgcagtgggtgcgccaggctcctggacagggcctggaatggatgggctggatcaacacccacagcggcgtgcccaaatacgccgaggacttcaagggcagagtgaccatcagcgccgacaccagcacctccacagcctacctgcagctgagcagcctgaagtccgaggacaccgccgtgtactactgcgccagaagcggcttcggcagcagctactggtacttcgacgtgtggggccagggcaccctcgtgaccgtcagctcagcctccaccaagggcccaagcgtcttccccctggcaccctcctccaagagcacctctggcggcacagccgccctgggctgcctggtcaaggactacttccccgaacccgtgaccgtgagctggaactcaggcgccctgaccagcggcgtgcacaccttccccgctgtcctgcagtcctcaggactctactccctcagcagcgtggtgaccgtgccctccagcagcttgggcacccagacctacatctgcaacgtgaatcacaagcccagcaacaccaaggtggacaagagagttgagcccaaatcttgtgacaaaactcacacatgcccaccctgcccagcacctgaactcctggggggaccctcagtcttcctcttccccccaaaacccaaggacaccctcatgatctcccggacccctgaggtcacatgcgtggtggtggacgtgagccacgaagaccctgaggtcaagttcaactggtacgtggacggcgtggaggtgcataatgccaagacaaagccccgggaggagcagtacaacagcacgtaccgggtggtcagcgtcctcaccgtcctgcaccaggactggctgaatggcaaggagtacaagtgcaaggtctccaacaaagccctcccagcccccatcgagaaaaccatctccaaagccaaaggccagccccgggaaccacaggtgtacaccctgcccccatcccgggaggagatgaccaagaaccaggtcagcctgacctgcctggtcaaaggcttctatcccagcgacatcgccgtggagtgggagagcaatggccagcccgagaacaactacaagaccacccctcccgtgctggactccgacggctccttcttcctctacagcaagctcaccgtggacaagagcaggtggcagcagggcaacgtcttctcatgctccgtgatgcatgaggctctgcacaaccactacacccagaagagcctctccctgtctcccggcaaa

SEQ ID NO: 2 - protein, 470 aa, synthetic construct
  REGION 1..470: note = Synthetic Construct
MKHLWFFLLLVAAPRWVLSQVQLVQSGAEVKKPGASVKVSCKASGYTFTTAGMQWVRQAPGQGLEWMGWINTHSGVPKYAEDFKGRVTISADTSTSTAYLQLSSLKSEDTAVYYCARSGFGSSYWYFDVWGQGTLVTVSSASTKGPSVFPLAPSSKSTSGGTAALGCLVKDYFPEPVTVSWNSGALTSGVHTFPAVLQSSGLYSLSSVVTVPSSSLGTQTYICNVNHKPSNTKVDKRVEPKSCDKTHTCPPCPAPELLGGPSVFLFPPKPKDTLMISRTPEVTCVVVDVSHEDPEVKFNWYVDGVEVHNAKTKPREEQYNSTYRVVSVLTVLHQDWLNGKEYKCKVSNKALPAPIEKTISKAKGQPREPQVYTLPPSREEMTKNQVSLTCLVKGFYPSDIAVEWESNGQPENNYKTTPPVLDSDGSFFLYSKLTVDKSRWQQGNVFSCSVMHEALHNHYTQKSLSLSPGK

SEQ ID NO: 3 - DNA, 702 bp, synthetic construct
  misc_feature 1..702: note = hTINA1-L1
  source 1..702: mol_type = other DNA
  CDS 1..702: protein_id = 4; translation = MVLQTQVFISLLLWISGAYGDIQMTQSPSSLSASVGDRVTITCKASQDVSTAVAWYQQKPGKAPKLLIYSASYRYTGVPSRFSGSGSGTDFTLTISSLQPEDFAVYYCQQHYITPLTFGQGTKLEIKRTVAAPSVFIFPPSDEQLKSGTASVVCLLNNFYPREAKVQWKVDNALQSGNSQESVTEQDSKDSTYSLSSTLTLSKADYEKHKVYACEVTHQGLSSPVTKSFNRGEC
atggtgctgcagacccaggtgttcatctccctgctgctgtggatctccggcgcgtacggcgacatccagatgacccagagccctagcagcctgagcgccagcgtgggcgacagagtgaccatcacatgcaaggccagccaggacgtgtccacagccgtggcctggtatcagcagaagcctggcaaggcccccaagctgctgatctacagcgccagctaccggtacaccggcgtgcccagcagattttctggcagcggctccggcaccgacttcaccctgacaatcagcagcctgcagcccgaggacttcgccgtgtactactgccagcagcactacatcacccccctgacctttggccagggcaccaagctggaaatcaagcgtacggtggccgccccctccgtgttcatcttccccccctccgacgagcagctgaagtccggcaccgcctccgtggtgtgcctgctgaataacttctaccccagagaggccaaggtgcagtggaaggtggacaacgccctgcagtccgggaactcccaggagagcgtgaccgagcaggacagcaaggacagcacctacagcctgagcagcaccctgaccctgagcaaagccgactacgagaagcacaaggtgtacgcctgcgaggtgacccaccagggcctgagctcccccgtcaccaagagcttcaacaggggggagtgt

SEQ ID NO: 4 - protein, 234 aa, synthetic construct
  REGION 1..234: note = Synthetic Construct
MVLQTQVFISLLLWISGAYGDIQMTQSPSSLSASVGDRVTITCKASQDVSTAVAWYQQKPGKAPKLLIYSASYRYTGVPSRFSGSGSGTDFTLTISSLQPEDFAVYYCQQHYITPLTFGQGTKLEIKRTVAAPSVFIFPPSDEQLKSGTASVVCLLNNFYPREAKVQWKVDNALQSGNSQESVTEQDSKDSTYSLSSTLTLSKADYEKHKVYACEVTHQGLSSPVTKSFNRGEC

SEQ ID NO: 5 - protein, 5 aa, Mus musculus
TAGMQ

SEQ ID NO: 6 - protein, 17 aa, Mus musculus
WINTHSGVPKYAEDFKG

SEQ ID NO: 7 - protein, 12 aa, Mus musculus
SGFGSSYWYFDV

SEQ ID NO: 8 - protein, 11 aa, Mus musculus
KASQDVSTAVA

SEQ ID NO: 9 - protein, 7 aa, Mus musculus
SASYRYT

SEQ ID NO: 10 - protein, 9 aa, Mus musculus
QQHYITPLT

SEQ ID NO: 11 - DNA, 1395 bp, synthetic construct
  misc_feature 1..1395: note = hM23-H1
  source 1..1395: mol_type = other DNA
  CDS 1..1395: protein_id = 12; translation = MKHLWFFLLLVAAPRWVLSQVQLVQSGAEVKKPGASVKVSCKASGYAFSNYLIEWVRQAPGQGLEWMGVINPGSGVTNYNEKFKGRVTITADTSTSTAYMELSSLRSEDTAVYYCARAEAWFAYWGQGTLVTVSSASTKGPSVFPLAPSSKSTSGGTAALGCLVKDYFPEPVTVSWNSGALTSGVHTFPAVLQSSGLYSLSSVVTVPSSSLGTQTYICNVNHKPSNTKVDKRVEPKSCDKTHTCPPCPAPELLGGPSVFLFPPKPKDTLMISRTPEVTCVVVDVSHEDPEVKFNWYVDGVEVHNAKTKPREEQYNSTYRVVSVLTVLHQDWLNGKEYKCKVSNKALPAPIEKTISKAKGQPREPQVYTLPPSREEMTKNQVSLTCLVKGFYPSDIAVEWESNGQPENNYKTTPPVLDSDGSFFLYSKLTVDKSRWQQGNVFSCSVMHEALHNHYTQKSLSLSPGK
atgaaacacctgtggttcttcctcctgctggtggcagctcccagatgggtgctgagccaggtgcagctggtgcagtctggcgccgaagtgaagaaaccaggcgccagcgtgaaggtgtcctgcaaggccagcggctacgccttcagcaactacctgatcgagtgggtgcgccaggcccctggacagggactggaatggatgggcgtgatcaaccctggcagcggcgtgaccaactacaacgagaagttcaagggcagagtgaccatcaccgccgacaccagcacctccaccgcctacatggaactgagcagcctgcggagcgaggacaccgccgtgtactattgtgccagagccgaggcttggtttgcctactggggccagggaaccctcgtgaccgtcagctcagcctccaccaagggcccaagcgtcttccccctggcaccctcctccaagagcacctctggcggcacagccgccctgggctgcctggtcaaggactacttccccgaacccgtgaccgtgagctggaactcaggcgccctgaccagcggcgtgcacaccttccccgctgtcctgcagtcctcaggactctactccctcagcagcgtggtgaccgtgccctccagcagcttgggcacccagacctacatctgcaacgtgaatcacaagcccagcaacaccaaggtggacaagagagttgagcccaaatcttgtgacaaaactcacacatgcccaccctgcccagcacctgaactcctggggggaccctcagtcttcctcttccccccaaaacccaaggacaccctcatgatctcccggacccctgaggtcacatgcgtggtggtggacgtgagccacgaagaccctgaggtcaagttcaactggtacgtggacggcgtggaggtgcataatgccaagacaaagccccgggaggagcagtacaacagcacgtaccgggtggtcagcgtcctcaccgtcctgcaccaggactggctgaatggcaaggagtacaagtgcaaggtctccaacaaagccctcccagcccccatcgagaaaaccatctccaaagccaaaggccagccccgggaaccacaggtgtacaccctgcccccatcccgggaggagatgaccaagaaccaggtcagcctgacctgcctggtcaaaggcttctatcccagcgacatcgccgtggagtgggagagcaatggccagcccgagaacaactacaagaccacccctcccgtgctggactccgacggctccttcttcctctacagcaagctcaccgtggacaagagcaggtggcagcagggcaacgtcttctcatgctccgtgatgcatgaggctctgcacaaccactacacccagaagagcctctccctgtctcccggcaaa

SEQ ID NO: 12 - protein, 465 aa, synthetic construct
  REGION 1..465: note = Synthetic Construct
MKHLWFFLLLVAAPRWVLSQVQLVQSGAEVKKPGASVKVSCKASGYAFSNYLIEWVRQAPGQGLEWMGVINPGSGVTNYNEKFKGRVTITADTSTSTAYMELSSLRSEDTAVYYCARAEAWFAYWGQGTLVTVSSASTKGPSVFPLAPSSKSTSGGTAALGCLVKDYFPEPVTVSWNSGALTSGVHTFPAVLQSSGLYSLSSVVTVPSSSLGTQTYICNVNHKPSNTKVDKRVEPKSCDKTHTCPPCPAPELLGGPSVFLFPPKPKDTLMISRTPEVTCVVVDVSHEDPEVKFNWYVDGVEVHNAKTKPREEQYNSTYRVVSVLTVLHQDWLNGKEYKCKVSNKALPAPIEKTISKAKGQPREPQVYTLPPSREEMTKNQVSLTCLVKGFYPSDIAVEWESNGQPENNYKTTPPVLDSDGSFFLYSKLTVDKSRWQQGNVFSCSVMHEALHNHYTQKSLSLSPGK

SEQ ID NO: 13 - DNA, 720 bp, synthetic construct
  misc_feature 1..720: note = hM23-L1
  source 1..720: mol_type = other DNA
  CDS 1..720: protein_id = 14; translation = MVLQTQVFISLLLWISGAYGDIVMTQSPDSLAVSLGERATINCKSSQSLLYSSNQKNYLAWYQQKPGQPPKLLIYWASTRESGVPDRFSGSGSGTDFTLTISSLQAEDVAVYYCQRYYGYPWTFGQGTKVEIKRTVAAPSVFIFPPSDEQLKSGTASVVCLLNNFYPREAKVQWKVDNALQSGNSQESVTEQDSKDSTYSLSSTLTLSKADYEKHKVYACEVTHQGLSSPVTKSFNRGEC
atggtgctgcagacccaggtgttcatctccctgctgctgtggatctccggcgcgtacggcgacatcgtgatgacccagagccctgacagcctggccgtgtctctgggagagagagccaccatcaactgcaagagcagccagagcctgctgtactccagcaaccagaagaactacctggcctggtatcagcagaagcccggccagcctcccaagctgctgatctactgggccagcaccagagaaagcggcgtgcccgatagattcagcggcagcggaagcggcaccgacttcaccctgacaatcagctccctgcaggccgaggacgtggccgtgtactactgccagcggtactacggctacccctggacctttggccagggcaccaaggtggaaatcaagcgtacggtggccgccccctccgtgttcatcttccccccctccgacgagcagctgaagtccggcaccgcctccgtggtgtgcctgctgaataacttctaccccagagaggccaaggtgcagtggaaggtggacaacgccctgcagtccgggaactcccaggagagcgtgaccgagcaggacagcaaggacagcacctacagcctgagcagcaccctgaccctgagcaaagccgactacgagaagcacaaggtgtacgcctgcgaggtgacccaccagggcctgagctcccccgtcaccaagagcttcaacaggggggagtgt

SEQ ID NO: 14 - protein, 240 aa, synthetic construct
  REGION 1..240: note = Synthetic Construct
MVLQTQVFISLLLWISGAYGDIVMTQSPDSLAVSLGERATINCKSSQSLLYSSNQKNYLAWYQQKPGQPPKLLIYWASTRESGVPDRFSGSGSGTDFTLTISSLQAEDVAVYYCQRYYGYPWTFGQGTKVEIKRTVAAPSVFIFPPSDEQLKSGTASVVCLLNNFYPREAKVQWKVDNALQSGNSQESVTEQDSKDSTYSLSSTLTLSKADYEKHKVYACEVTHQGLSSPVTKSFNRGEC

SEQ ID NO: 15 - protein, 5 aa, Mus musculus
NYLIE

SEQ ID NO: 16 - protein, 17 aa, Mus musculus
VINPGSGVTNYNEKFKG

SEQ ID NO: 17 - protein, 7 aa, Mus musculus
AEAWFAY

SEQ ID NO: 18 - protein, 17 aa, Mus musculus
KSSQSLLYSSNQKNYLA

SEQ ID NO: 19 - protein, 7 aa, Mus musculus
WASTRES

SEQ ID NO: 20 - protein, 9 aa, Mus musculus
QRYYGYPWT

SEQ ID NO: 21 - DNA, 22 bp, synthetic construct
  misc_feature 1..22: note = primer EG-Inf-F
  source 1..22: mol_type = other DNA
agctcccagatgggtgctgagc

SEQ ID NO: 22 - DNA, 22 bp, synthetic construct
  misc_feature 1..22: note = primer EG1-Inf-R
  source 1..22: mol_type = other DNA
gggcccttggtggaggctgagc

SEQ ID NO: 23 - DNA, 24 bp, synthetic construct
  misc_feature 1..24: note = primer CM-LKF
  source 1..24: mol_type = other DNA
ctgtggatctccggcgcgtacggc

SEQ ID NO: 24 - DNA, 21 bp, synthetic construct
  misc_feature 1..21: note = primer KCL-Inf-R
  source 1..21: mol_type = other DNA
ggagggggcggccaccgtacg

SEQ ID NO: 25 - protein, 471 aa, synthetic construct
  REGION 1..471: note = M30-H1
MKHLWFFLLLVAAPRWVLSQVQLVQSGAEVKKPGSSVKVSCKASGYTFTNYVMHWVRQAPGQGLEWMGYINPYNDDVKYNEKFKGRVTITADESTSTAYMELSSLRSEDTAVYYCARWGYYGSPLYYFDYWGQGTLVTVSSASTKGPSVFPLAPSSKSTSGGTAALGCLVKDYFPEPVTVSWNSGALTSGVHTFPAVLQSSGLYSLSSVVTVPSSSLGTQTYICNVNHKPSNTKVDKRVEPKSCDKTHTCPPCPAPELLGGPSVFLFPPKPKDTLMISRTPEVTCVVVDVSHEDPEVKFNWYVDGVEVHNAKTKPREEQYNSTYRVVSVLTVLHQDWLNGKEYKCKVSNKALPAPIEKTISKAKGQPREPQVYTLPPSREEMTKNQVSLTCLVKGFYPSDIAVEWESNGQPENNYKTTPPVLDSDGSFFLYSKLTVDKSRWQQGNVFSCSVMHEALHNHYTQKSLSLSPGK

SEQ ID NO: 26 - protein, 233 aa, synthetic construct
  REGION 1..233: note = M30-L4
MVLQTQVFISLLLWISGAYGEIVLTQSPATLSLSPGERATLSCRASSRLIYMHWYQQKPGQAPRPLIYATSNLASGIPARFSGSGSGTDFTLTISSLEPEDFAVYYCQQWNSNPPTFGQGTKVEIKRTVAAPSVFIFPPSDEQLKSGTASVVCLLNNFYPREAKVQWKVDNALQSGNSQESVTEQDSKDSTYSLSSTLTLSKADYEKHKVYACEVTHQGLSSPVTKSFNRGEC

SEQ ID NO: 27 - protein, 5 aa, Mus musculus
NYVMH

SEQ ID NO: 28 - protein, 17 aa, Mus musculus
YINPYNDDVKYNEKFKG

SEQ ID NO: 29 - protein, 13 aa, Mus musculus
WGYYGSPLYYFDY

SEQ ID NO: 30 - protein, 10 aa, Mus musculus
RASSRLIYMH

SEQ ID NO: 31 - protein, 7 aa, Mus musculus
ATSNLAS

SEQ ID NO: 32 - protein, 9 aa, Mus musculus
QQWNSNPPT

SEQ ID NO: 33 - protein, 450 aa, synthetic construct
  REGION 1..450: note = Heavy chain of Trastuzumab
EVQLVESGGGLVQPGGSLRLSCAASGFNIKDTYIHWVRQAPGKGLEWVARIYPTNGYTRYADSVKGRFTISADTSKNTAYLQMNSLRAEDTAVYYCSRWGGDGFYAMDYWGQGTLVTVSSASTKGPSVFPLAPSSKSTSGGTAALGCLVKDYFPEPVTVSWNSGALTSGVHTFPAVLQSSGLYSLSSVVTVPSSSLGTQTYICNVNHKPSNTKVDKKVEPKSCDKTHTCPPCPAPELLGGPSVFLFPPKPKDTLMISRTPEVTCVVVDVSHEDPEVKFNWYVDGVEVHNAKTKPREEQYNSTYRVVSVLTVLHQDWLNGKEYKCKVSNKALPAPIEKTISKAKGQPREPQVYTLPPSREEMTKNQVSLTCLVKGFYPSDIAVEWESNGQPENNYKTTPPVLDSDGSFFLYSKLTVDKSRWQQGNVFSCSVMHEALHNHYTQKSLSLSPGK

SEQ ID NO: 34 - protein, 214 aa, synthetic construct
  REGION 1..214: note = Light chain of Trastuzumab
DIQMTQSPSSLSASVGDRVTITCRASQDVNTAVAWYQQKPGKAPKLLIYSASFLYSGVPSRFSGSRSGTDFTLTISSLQPEDFATYYCQQHYTTPPTFGQGTKVEIKRTVAAPSVFIFPPSDEQLKSGTASVVCLLNNFYPREAKVQWKVDNALQSGNSQESVTEQDSKDSTYSLSSTLTLSKADYEKHKVYACEVTHQGLSSPVTKSFNRGEC